European Patent Specification EP 4 010 492 B1, published April 15, 2026. Title: LOGIC DRIVEN POLYNUCLEOTIDE SCANNING FOR MAPPING FEATURES IN A NANOPORE DEVICE. Applicant: Ontera Inc Dunbar, William Xu, Liu. The sequence listing filed with the application follows.

SEQUENCE LISTING (1 sequence)

SEQ ID NO: 1 - DNA, 90 bp, Artificial Sequence
  Synthetic sequence
aaaaaaaaaagggaaagggaaagggaaagaaaaaaaaaaaaaaaaaaaagggaaagggaaaaaaaaaagagagagagagagagagaagag